European Patent Application EP 4 249 596 A1, published September 27, 2023. Title: A novel transgenic vaccinia virus and use of the virus. Applicant: National University Corporation Tottori University. The sequence listing filed with the application follows.

SEQUENCE LISTING (16 sequences)

SEQ ID NO: 1 - DNA, 37 bp, Artificial
  Primer
atggccggaccggccaccggtcgccaccatgagcgag

SEQ ID NO: 2 - DNA, 41 bp, Artificial
  Primer
tcgaattcgctagcggccgcttaattaagcttgtgccccag

SEQ ID NO: 3 - DNA, 20 bp, Artificial
  Primer
acagggattaagacggaaag

SEQ ID NO: 4 - DNA, 20 bp, Artificial
  Primer
gtcaacaagcatcttccaac

SEQ ID NO: 5 - DNA, 605 bp, encephalomyocarditis virus
tgcatctagggcggccaattccgcccctctccctcccccccccctaacgttactggccgaagccgcttggaataaggccggtgtgcgtttgtctatatgtgattttccaccatattgccgtcttttggcaatgtgagggcccggaaacctggccctgtcttcttgacgagcattcctaggggtctttcccctctcgccaaaggaatgcaaggtctgttgaatgtcgtgaaggaagcagttcctctggaagcttcttgaagacaaacaacgtctgtagcgaccctttgcaggcagcggaaccccccacctggcgacaggtgcctctgcggccaaaagccacgtgtataagatacacctgcaaaggcggcacaaccccagtgccacgttgtgagttggatagttgtggaaagagtcaaatggctctcctcaagcgtattcaacaaggggctgaaggatgcccagaaggtaccccattgtatgggatctgatctggggcctcggtgcacatgctttacatgtgtttagtcgaggttaaaaaaacgtctaggccccccgaaccacggggacgtggttttcctttgaaaaacacgatgataagcttgcca

SEQ ID NO: 6 - protein, 335 aa, Mus musculus
MCPQKLTISWFAIVLLVSPLMAMWELEKDVYVVEVDWTPDAPGETVNLTCDTPEEDDITWTSDQRHGVIGSGKTLTITVKEFLDAGQYTCHKGGETLSHSHLLLHKKENGIWSTEILKNFKNKTFLKCEAPNYSGRFTCSWLVQRNMDLKFNIKSSSSSPDSRAVTCGMASLSAEKVTLDQRDYEKYSVSCQEDVTCPTAEETLPIELALEARQQNKYENYSTSFFIRDIIKPDPPKNLQMKPLKNSQVEVSWEYPDSWSTPHSYFSLKFFVRIQRKKEKMKETEEGCNQKGAFLVEKTSTEVQCKGGNVCVQAQDRYYNSSCSKWACVPCRVRS

SEQ ID NO: 7 - protein, 236 aa, Mus musculus
MVSVPTASPSASSSSSQCRSSMCQSRYLLFLATLALLNHLSLARVIPVSGPARCLSQSRNLLKTTDDMVKTAREKLKHYSCTAEDIDHEDITRDQTSTLKTCLPLELHKNESCLATRETSSTTRGSCLPPQKTSLMMTLCLGSIYEDLKMYQTEFQAINAALQNHNHQQIILDKGMLVAIDELMQSLNHNGETLRQKPPVGEADPYRVKMKLCILLHAFSTRVVTINRVMGYLSSA

SEQ ID NO: 8 - protein, 177 aa, Homo sapiens
MFHVSFRYIFGLPPLILVLLPVASSDCDIEGKDGKQYESVLMVSIDQLLDSMKEIGSNCLNNEFNFFKRHICDANKEGMFLFRAARKLRQFLKMNSTGDFDLHLLKVSEGTTILLNCTGQVKGRKPAALGEAQPTKSLEENKSLKEQKKLNDLCFLKRLLQEIKTCWNKILMGTKEH

SEQ ID NO: 9 - protein, 133 aa, Mus musculus
MAQMMTLSLLSLVLALCIPWTQGSDGGGQDCCLKYSQKKIPYSIVRGYRKQEPSLGCPIPAILFSPRKHSKPELCANPEEGWVQNLMRRLDQPPAPGKQSPGCRKNRGTSKSGKKGKGSKGCKRTEQTQPSRG

SEQ ID NO: 10 - DNA, 20 bp, Artificial
  Primer
ggtaacgctatcgaaacgac

SEQ ID NO: 11 - DNA, 20 bp, Artificial
  Primer
ttagttcgtcgagtgaacct

SEQ ID NO: 12 - DNA, 20 bp, Artificial
  Primer
acagggattaagacggaaag

SEQ ID NO: 13 - DNA, 20 bp, Artificial
  Primer
gtcaacaagcatcttccaac

SEQ ID NO: 14 - protein, 260 aa, Mus musculus
MIETYSQPSPRSVATGLPASMKIFMYLLTVFLITQMIGSVLFAVYLHRRLDKVEEEVNLHEDFVFIKKLKRCNKGEGSLSLLNCEEMRRQFEDLVKDITLNKEEKKENSFEMQRGDEDPQIAAHVVSEANSNAASVLQWAKKGYYTMKSNLVMLENGKQLTVKREGLYYVYTQVTFCSNREPSSQRPFIVGLWLKPSSGSERILLKAANTHSSSQLCEQQSVHLGGVFELQAGASVFVNVTEASQVIHRVGFSSFGLLKL

SEQ ID NO: 15 - DNA, 1110 bp, Vaccinia virus
atgattgcgttattgatactatcgttagcgtgttcagcgtccgcctatcgtctacaaggatttaccaatgccggtatagtagcgtataaaaatattcaagatgataatattgtcttctcaccgtttggttattcgttttctatgtttatgtcgctattgcctgcatcaggtaatactagaatagaattattgaagactatggatttgagaaaaagagatctgggtccagcatttacagaattaatatcaggattagctaagctgaaaacatctaaatatacgtacactgatctaacttatcaaagtttcgtagataatactgtgtgtattaaaccgtcgtattatcaacaatatcatagattcggcctatatagattaaactttagacgagatgcggttaataaaattaattctatagtagaacgtagatccggtatgtctaatgtagtagattctaatatgctcgacaataatactctatgggcaatcattaatactatatattttaaaggtatatggcaatatccgtttgatatcactaaaacacgcaatgctagttttactaataagtacggtacgaaaacggttcccatgatgaacgtagttactaaattgcaaggaaatacaatcacaatcgatgacaaagaatatgacatggtacgccttccgtataaggatgctaatattagtatgtacctggcaataggtgataatatgacccatttcacagattctatcacggctgcaaaattagactattggtcgtttcaattagggaataaagtgtacaatcttaaactccctaaattttctatcgaaaataagagggatattaagtcgatagccgaaatgatggctcctagtatgtttaatccagataatgcgtcgtttaaacatatgactagggacccattatatatttataaaatgtttcagaatgcaaagatagatgtcgacgaacaaggaactgtagcagaggcatctactattatggtagctacggcgagatcatctcctgaaaaactggaatttaatacaccatttgtgttcatcatcagacatgatattactggatttatattgtttatgggtaaggtggaatctccttaa

SEQ ID NO: 16 - DNA, 933 bp, Vaccinia virus
atgacacgattaccaatacttttgttactaatatcattagtatacgctacaccttctcctcagacatctaaaaaaataggtgatgatgcaactctatcatgtaatcgaaataatacaaatgactacgttgttatgagtgcttggtataaggagcccaattccattattcttttagctgctaaaagcgacgtcttgtattttgataattataccaaggataaaatatcttacgactctccatacgatgatctagttacaactatcacaattaaatcattgactgctagagatgccggtacttatgtatgtgcattctttatgacatcgcctacaaatgacactgataaagtagattatgaagaatactccacagagttgattgtaaatacagatagtgaatcgactatagacataatactatctggatctacacattcaccggaaactagttctgagaaacctgattatatagataattctaattgctcgtcggtattcgaaatcgcgactccggaaccaattactgataatgtagaagatcatacagacaccgtcacatacactagtgatagcattaatacagtaagtgcatcatctggagaatccacaacagacgagactccggaaccaattactgataaagaagaagatcatacagtcacagacactgtctcatacactacagtaagtacatcatctggaattgtcactactaaatcaaccaccgatgatacgtacaatgataatgatacagtaccaccaactactgtaggcggtagtacaacctctattagcaattataaaaccaaggactttgtagaaatatttggtattaccgcattaattatattgtcggccgtggcaatattctgtattacgtattatatatgtaataaacgttcacgtaaatacaaaacagagaacaaagtctag